European Patent Application EP 4 245 311 A1, published September 20, 2023. Title: Use of an enzyme fusion protein for prevention or treatment of renal disease. Applicant: HANMI PHARM. CO., LTD. The sequence listing filed with the application follows.

SEQUENCE LISTING (31 sequences)

SEQ ID NO: 1 - DNA, 43 bp, Artificial Sequence
  Fc(S2P)_F
ctggcggtggcggatcgccaccatgcccagcacctgagttcct

SEQ ID NO: 2 - DNA, 43 bp, Artificial Sequence
  Fc(S2P)_R
aggaactcaggtgctgggcatggtggcgatccgccaccgccag

SEQ ID NO: 3 - DNA, 43 bp, Artificial Sequence
  Fc(N71Q)_F
agccgcgggaggagcagttccaaagcacgtaccgtgtggtcag

SEQ ID NO: 4 - DNA, 43 bp, Artificial Sequence
  Fc(N71Q)_R
ctgaccacacggtacgtgctttggaactgctcctcccgcggct

SEQ ID NO: 5 - DNA, 1287 bp, Homo sapiens
atgcagctgaggaacccagaactacatctgggctgcgcgcttgcgcttcgcttcctggccctcgtttcctgggacatccctggggctagagcactggacaatggattggcaaggacgcctaccatgggctggctgcactgggagcgcttcatgtgcaaccttgactgccaggaagagccagattcctgcatcagtgagaagctcttcatggagatggcagagctcatggtctcagaaggctggaaggatgcaggttatgagtacctctgcattgatgactgttggatggctccccaaagagattcagaaggcagacttcaggcagaccctcagcgctttcctcatgggattcgccagctagctaattatgttcacagcaaaggactgaagctagggatttatgcagatgttggaaataaaacctgcgcaggcttccctgggagttttggatactacgacattgatgcccagacctttgctgactggggagtagatctgctaaaatttgatggttgttactgtgacagtttggaaaatttggcagatggttataagcacatgtccttggccctgaataggactggcagaagcattgtgtactcctgtgagtggcctctttatatgtggccctttcaaaagcccaattatacagaaatccgacagtactgcaatcactggcgaaattttgctgacattgatgattcctggaaaagtataaagagtatcttggactggacatcttttaaccaggagagaattgttgatgttgctggaccagggggttggaatgacccagatatgttagtgattggcaactttggcctcagctggaatcagcaagtaactcagatggccctctgggctatcatggctgctcctttattcatgtctaatgacctccgacacatcagccctcaagccaaagctctccttcaggataaggacgtaattgccatcaatcaggaccccttgggcaagcaagggtaccagcttagacagggagacaactttgaagtgtgggaacgacctctctcaggcttagcctgggctgtagctatgataaaccggcaggagattggtggacctcgctcttataccatcgcagttgcttccctgggtaaaggagtggcctgtaatcctgcctgcttcatcacacagctcctccctgtgaaaaggaagctagggttctatgaatggacttcaaggttaagaagtcacataaatcccacaggcactgttttgcttcagctagaaaatacaatgcagatgtcattaaaagacttactt

SEQ ID NO: 6 - protein, 429 aa, Homo sapiens
MQLRNPELHLGCALALRFLALVSWDIPGARALDNGLARTPTMGWLHWERFMCNLDCQEEPDSCISEKLFMEMAELMVSEGWKDAGYEYLCIDDCWMAPQRDSEGRLQADPQRFPHGIRQLANYVHSKGLKLGIYADVGNKTCAGFPGSFGYYDIDAQTFADWGVDLLKFDGCYCDSLENLADGYKHMSLALNRTGRSIVYSCEWPLYMWPFQKPNYTEIRQYCNHWRNFADIDDSWKSIKSILDWTSFNQERIVDVAGPGGWNDPDMLVIGNFGLSWNQQVTQMALWAIMAAPLFMSNDLRHISPQAKALLQDKDVIAINQDPLGKQGYQLRQGDNFEVWERPLSGLAWAVAMINRQEIGGPRSYTIAVASLGKGVACNPACFITQLLPVKRKLGFYEWTSRLRSHINPTGTVLLQLENTMQMSLKDLL

SEQ ID NO: 7 - DNA, 666 bp, Artificial Sequence
  Fc varinat
ccaccatgcccagcacctgagttcctggggggaccatcagtcttcctgttccccccaaaacccaaggacaccctcatgatctcccggacccctgaggtcacatgcgtggtggtggacgtgagccaggaagaccctgaggtccagttcaactggtacgtggacggcgtggaggtgcataatgccaagacaaagccgcgggaggagcagttccaaagcacgtaccgtgtggtcagcgtcctcaccgtcctgcaccaggactggctgaatggcaaggagtacaagtgcaaggtctccaacaaaggcctcccatcctccatcgagaaaaccatctccaaagccaaagggcagccccgagaaccacaggtgtacaccctgcccccatcccaggaggagatgaccaagaaccaggtcagcctgacctgcctggtcaaaggcttctatcccagcgacatcgccgtggagtgggagagcaatgggcagccggagaacaactacaagaccacgcctcccgtgctggactccgacggctccttcttcctctacagcaggctaaccgtggacaagagcaggtggcaggaggggaacgtcttctcatgctccgtgatgcatgaggctctgcacaaccactacacgcagaagagcctctccctgtctctgggtaaatga

SEQ ID NO: 8 - protein, 221 aa, Artificial Sequence
  Fc variant
PSCPAPEFLGGPSVFLFPPKPKDTLMISRTPEVTCVVVDVSQEDPEVQFNWYVDGVEVHNAKTKPREEQFNSTYRVVSVLTVLHQDWLNGKEYKCKVSNKGLPSSIEKTISKAKGQPREPQVYTLPPSQEEMTKNQVSLTCLVKGFYPSDIAVEWESNGQPENNYKTTPPVLDSDGSFFLYSRLTVDKSRWQEGNVFSCSVMHEALHNHYTQKSLSLSLGK

SEQ ID NO: 9 - protein, 221 aa, Artificial Sequence
  Fc varinat
PPCPAPEFLGGPSVFLFPPKPKDTLMISRTPEVTCVVVDVSQEDPEVQFNWYVDGVEVHNAKTKPREEQFQSTYRVVSVLTVLHQDWLNGKEYKCKVSNKGLPSSIEKTISKAKGQPREPQVYTLPPSQEEMTKNQVSLTCLVKGFYPSDIAVEWESNGQPENNYKTTPPVLDSDGSFFLYSRLTVDKSRWQEGNVFSCSVMHEALHNHYTQKSLSLSLGK

SEQ ID NO: 10 - DNA, 90 bp, Artificial Sequence
  peptide linker
ggcggcggaggttcaggtggtggtggctctggcggtggagggtcggggggaggcggctctggaggagggggctccggtgggggaggtagc

SEQ ID NO: 11 - protein, 30 aa, Artificial Sequence
  peptide linker
GGGGSGGGGSGGGGSGGGGSGGGGSGGGGS

SEQ ID NO: 12 - DNA, 2043 bp, Artificial Sequence
  alpha galactosidase-Fc fusion protein
atgcagctgaggaacccagaactacatctgggctgcgcgcttgcgcttcgcttcctggccctcgtttcctgggacatccctggggctagagcactggacaatggattggcaaggacgcctaccatgggctggctgcactgggagcgcttcatgtgcaaccttgactgccaggaagagccagattcctgcatcagtgagaagctcttcatggagatggcagagctcatggtctcagaaggctggaaggatgcaggttatgagtacctctgcattgatgactgttggatggctccccaaagagattcagaaggcagacttcaggcagaccctcagcgctttcctcatgggattcgccagctagctaattatgttcacagcaaaggactgaagctagggatttatgcagatgttggaaataaaacctgcgcaggcttccctgggagttttggatactacgacattgatgcccagacctttgctgactggggagtagatctgctaaaatttgatggttgttactgtgacagtttggaaaatttggcagatggttataagcacatgtccttggccctgaataggactggcagaagcattgtgtactcctgtgagtggcctctttatatgtggccctttcaaaagcccaattatacagaaatccgacagtactgcaatcactggcgaaattttgctgacattgatgattcctggaaaagtataaagagtatcttggactggacatcttttaaccaggagagaattgttgatgttgctggaccagggggttggaatgacccagatatgttagtgattggcaactttggcctcagctggaatcagcaagtaactcagatggccctctgggctatcatggctgctcctttattcatgtctaatgacctccgacacatcagccctcaagccaaagctctccttcaggataaggacgtaattgccatcaatcaggaccccttgggcaagcaagggtaccagcttagacagggagacaactttgaagtgtgggaacgacctctctcaggcttagcctgggctgtagctatgataaaccggcaggagattggtggacctcgctcttataccatcgcagttgcttccctgggtaaaggagtggcctgtaatcctgcctgcttcatcacacagctcctccctgtgaaaaggaagctagggttctatgaatggacttcaaggttaagaagtcacataaatcccacaggcactgttttgcttcagctagaaaatacaatgcagatgtcattaaaagacttacttggcggcggaggttcaggtggtggtggctctggcggtggagggtcggggggaggcggctctggaggagggggctccggtgggggaggtagcccaccatgcccagcacctgagttcctggggggaccatcagtcttcctgttccccccaaaacccaaggacaccctcatgatctcccggacccctgaggtcacatgcgtggtggtggacgtgagccaggaagaccctgaggtccagttcaactggtacgtggacggcgtggaggtgcataatgccaagacaaagccgcgggaggagcagttccaaagcacgtaccgtgtggtcagcgtcctcaccgtcctgcaccaggactggctgaatggcaaggagtacaagtgcaaggtctccaacaaaggcctcccatcctccatcgagaaaaccatctccaaagccaaagggcagccccgagaaccacaggtgtacaccctgcccccatcccaggaggagatgaccaagaaccaggtcagcctgacctgcctggtcaaaggcttctatcccagcgacatcgccgtggagtgggagagcaatgggcagccggagaacaactacaagaccacgcctcccgtgctggactccgacggctccttcttcctctacagcaggctaaccgtggacaagagcaggtggcaggaggggaacgtcttctcatgctccgtgatgcatgaggctctgcacaaccactacacgcagaagagcctctccctgtctctgggtaaatga

SEQ ID NO: 13 - protein, 680 aa, Artificial Sequence
  alpha galactosidase-Fc fusion protein
MQLRNPELHLGCALALRFLALVSWDIPGARALDNGLARTPTMGWLHWERFMCNLDCQEEPDSCISEKLFMEMAELMVSEGWKDAGYEYLCIDDCWMAPQRDSEGRLQADPQRFPHGIRQLANYVHSKGLKLGIYADVGNKTCAGFPGSFGYYDIDAQTFADWGVDLLKFDGCYCDSLENLADGYKHMSLALNRTGRSIVYSCEWPLYMWPFQKPNYTEIRQYCNHWRNFADIDDSWKSIKSILDWTSFNQERIVDVAGPGGWNDPDMLVIGNFGLSWNQQVTQMALWAIMAAPLFMSNDLRHISPQAKALLQDKDVIAINQDPLGKQGYQLRQGDNFEVWERPLSGLAWAVAMINRQEIGGPRSYTIAVASLGKGVACNPACFITQLLPVKRKLGFYEWTSRLRSHINPTGTVLLQLENTMQMSLKDLLGGGGSGGGGSGGGGSGGGGSGGGGSGGGGSPPCPAPEFLGGPSVFLFPPKPKDTLMISRTPEVTCVVVDVSQEDPEVQFNWYVDGVEVHNAKTKPREEQFQSTYRVVSVLTVLHQDWLNGKEYKCKVSNKGLPSSIEKTISKAKGQPREPQVYTLPPSQEEMTKNQVSLTCLVKGFYPSDIAVEWESNGQPENNYKTTPPVLDSDGSFFLYSRLTVDKSRWQEGNVFSCSVMHEALHNHYTQKSLSLSLGK

SEQ ID NO: 14 - protein, 12 aa, Homo sapiens
ESKYGPPCPSCP

SEQ ID NO: 15 - DNA, 24 bp, Artificial Sequence
  TNF-a_F
gatctcaaagacaaccaacatgtg

SEQ ID NO: 16 - DNA, 24 bp, Artificial Sequence
  TNF-a_R
ctccagctggaagactcctcccag

SEQ ID NO: 17 - DNA, 20 bp, Artificial Sequence
  IL-6_F
ccagttgccttcttgggact

SEQ ID NO: 18 - DNA, 21 bp, Artificial Sequence
  IL-6_R
ggtctgttgggagtggtatcc

SEQ ID NO: 19 - DNA, 20 bp, Artificial Sequence
  RANTES_F
cctcaccatatggctcggac

SEQ ID NO: 20 - DNA, 20 bp, Artificial Sequence
  RANTES_R
acgactgcaagattggagca

SEQ ID NO: 21 - DNA, 21 bp, Artificial Sequence
  18s_F
taacgaacgagactctggcat

SEQ ID NO: 22 - DNA, 22 bp, Artificial Sequence
  18s_R
cggacatctaagggcatcacag

SEQ ID NO: 23 - DNA, 22 bp, Artificial Sequence
  TIMP-1_F
ccttgcaaactggagagtgaca

SEQ ID NO: 24 - DNA, 21 bp, Artificial Sequence
  TIMP-1_R
aggcaaagtgatcgctctggt

SEQ ID NO: 25 - DNA, 20 bp, Artificial Sequence
  Col1a1_F
ccttcttgaggttgccagtc

SEQ ID NO: 26 - DNA, 20 bp, Artificial Sequence
  Col1a1_R
agagcatgaccgatggattc

SEQ ID NO: 27 - DNA, 22 bp, Artificial Sequence
  a-SMA_F
gtgacatcgacatcaggaaaga

SEQ ID NO: 28 - DNA, 20 bp, Artificial Sequence
  a-SMA_R
gatccacatctgctggaagg

SEQ ID NO: 29 - DNA, 21 bp, Artificial Sequence
  18s_F
taacgaacgagactctggcat

SEQ ID NO: 30 - DNA, 22 bp, Artificial Sequence
  18s_R
cggacatctaagggcatcacag

SEQ ID NO: 31 - protein, 4 aa, Artificial Sequence
  Hinge region
PPCP